European Patent Application EP 4 260 863 A1, published October 18, 2023. Title: Composition for Preventive or Treatment of Neurological or Psychiatric Diseases Comprising Extracellular Vesicles Derived from Sphingomonas bacteria. Applicant: MD Healthcare Inc. The sequence listing filed with the application follows.

SEQUENCE LISTING (26 sequences)

SEQ ID NO: 1 - DNA, 20 bp, Artificial Sequence
  total Bdnf_F
tggctgacacttttgagcac

SEQ ID NO: 2 - DNA, 20 bp, Artificial Sequence
  total Bdnf_R
gtttgcggcatccaggtaat

SEQ ID NO: 3 - DNA, 19 bp, Artificial Sequence
  NT3_F
tactacggcaacagagacg

SEQ ID NO: 4 - DNA, 19 bp, Artificial Sequence
  NT3_R
gttgcccacataatcctcc

SEQ ID NO: 5 - DNA, 20 bp, Artificial Sequence
  NT4/5_F
ggctccatcctgaacatcat

SEQ ID NO: 6 - DNA, 20 bp, Artificial Sequence
  NT4/5_R
gccatgatctacctgcctgt

SEQ ID NO: 7 - DNA, 18 bp, Artificial Sequence
  Ngf_F
agcattcccttgacacag

SEQ ID NO: 8 - DNA, 18 bp, Artificial Sequence
  Ngf_R
ggtctacagtgatgttgc

SEQ ID NO: 9 - DNA, 22 bp, Artificial Sequence
  TrkB_F
aaggactttcatcgggaagctg

SEQ ID NO: 10 - DNA, 19 bp, Artificial Sequence
  TrkB_R
tcgccctccacacagacac

SEQ ID NO: 11 - DNA, 20 bp, Artificial Sequence
  HDAC1_F
cagtgtggctcagattccct

SEQ ID NO: 12 - DNA, 20 bp, Artificial Sequence
  HDAC1_R
gggcagctcattagggatct

SEQ ID NO: 13 - DNA, 20 bp, Artificial Sequence
  HDAC2_F
gggacaggcttggttgtttc

SEQ ID NO: 14 - DNA, 20 bp, Artificial Sequence
  HDAC2_R
gagcatcagcaatggcaagt

SEQ ID NO: 15 - DNA, 20 bp, Artificial Sequence
  HDAC3_F
agagaggtcccgaggagaac

SEQ ID NO: 16 - DNA, 20 bp, Artificial Sequence
  HDAC3_R
actcttggggacacagcatc

SEQ ID NO: 17 - DNA, 20 bp, Artificial Sequence
  HDAC4_F
caatcccacagtctccgtgt

SEQ ID NO: 18 - DNA, 20 bp, Artificial Sequence
  HDAC4_R
cagcaccccactaaggttca

SEQ ID NO: 19 - DNA, 20 bp, Artificial Sequence
  HDAC5_F
tgtcaccgccagatgttttg

SEQ ID NO: 20 - DNA, 20 bp, Artificial Sequence
  HDAC5_R
tgagcagagccgagacacag

SEQ ID NO: 21 - DNA, 21 bp, Artificial Sequence
  Sirt1_F
gatccttcagtgtcatggttc

SEQ ID NO: 22 - DNA, 18 bp, Artificial Sequence
  Sirt1_R
atggcaagtggctcatca

SEQ ID NO: 23 - DNA, 22 bp, Artificial Sequence
  Sirt5_F
atcgcaaggctggcaccaagaa

SEQ ID NO: 24 - DNA, 22 bp, Artificial Sequence
  Sirt5_R
ctaaagctgggcagatcggact

SEQ ID NO: 25 - DNA, 20 bp, Artificial Sequence
  Sirt7_F
gagagcgaggatctggtgac

SEQ ID NO: 26 - DNA, 20 bp, Artificial Sequence
  Sirt7_R
cgtgtagacaaccaagtgcc